European Patent Application EP 4 763 979 A1, published June 24, 2026. Title: 体内半衰期延长的工程化T细胞及其制备方法. Applicant: 博雅缉因（北京）生物科技有限公司. Application CN. The sequence listing filed with the application follows.

SEQUENCE LISTING (316 sequences)

SEQ ID NO: 1 - DNA, 20 bp, synthetic construct
  source 1..20: mol_type = other DNA
gctggtacacggcagggtca

SEQ ID NO: 2 - DNA, 20 bp, synthetic construct
  source 1..20: mol_type = other DNA
ctctcagctggtacacggca

SEQ ID NO: 3 - DNA, 20 bp, synthetic construct
  source 1..20: mol_type = other DNA
atttgtttgagaatcaaaat

SEQ ID NO: 4 - DNA, 20 bp, synthetic construct
  source 1..20: mol_type = other DNA
tctctcagctggtacacggc

SEQ ID NO: 5 - DNA, 20 bp, synthetic construct
  source 1..20: mol_type = other DNA
gagtagcgcgagcacagcta

SEQ ID NO: 6 - DNA, 20 bp, synthetic construct
  source 1..20: mol_type = other DNA
agcaagcaagcaccggaccc

SEQ ID NO: 7 - DNA, 20 bp, synthetic construct
  source 1..20: mol_type = other DNA
ggcggcggcgcggagaacaa

SEQ ID NO: 8 - DNA, 20 bp, synthetic construct
  source 1..20: mol_type = other DNA
gccatggcgctgcctctcgt

SEQ ID NO: 9 - DNA, 20 bp, synthetic construct
  source 1..20: mol_type = other DNA
cactcgatcacacccgccga

SEQ ID NO: 10 - DNA, 20 bp, synthetic construct
  source 1..20: mol_type = other DNA
ggggcgggcgaacggcaaga

SEQ ID NO: 11 - DNA, 20 bp, synthetic construct
  source 1..20: mol_type = other DNA
cggcggcggcgggctcgctc

SEQ ID NO: 12 - DNA, 20 bp, synthetic construct
  source 1..20: mol_type = other DNA
cctgcagcggagcccacgag

SEQ ID NO: 13 - DNA, 20 bp, synthetic construct
  source 1..20: mol_type = other DNA
gggcgggcgaacggcaagac

SEQ ID NO: 14 - DNA, 20 bp, synthetic construct
  source 1..20: mol_type = other DNA
tcttgccgttcgcccgcccc

SEQ ID NO: 15 - DNA, 20 bp, synthetic construct
  source 1..20: mol_type = other DNA
gcggcggcgcggagaacaag

SEQ ID NO: 16 - DNA, 20 bp, synthetic construct
  source 1..20: mol_type = other DNA
gccccgcgcgcagtgagcgc

SEQ ID NO: 17 - DNA, 20 bp, synthetic construct
  source 1..20: mol_type = other DNA
ctggctcgctggctgcacgg

SEQ ID NO: 18 - DNA, 20 bp, synthetic construct
  source 1..20: mol_type = other DNA
cggcggcgcggagaacaagg

SEQ ID NO: 19 - DNA, 20 bp, synthetic construct
  source 1..20: mol_type = other DNA
ccactcgatcacacccgccg

SEQ ID NO: 20 - DNA, 20 bp, synthetic construct
  source 1..20: mol_type = other DNA
cccggccgcgccttcagcta

SEQ ID NO: 21 - DNA, 20 bp, synthetic construct
  source 1..20: mol_type = other DNA
ctctcggcctccctcacccg

SEQ ID NO: 22 - DNA, 20 bp, synthetic construct
  source 1..20: mol_type = other DNA
gaggggggcgctaggcgatg

SEQ ID NO: 23 - DNA, 20 bp, synthetic construct
  source 1..20: mol_type = other DNA
ggagaggccgggctccgaag

SEQ ID NO: 24 - DNA, 20 bp, synthetic construct
  source 1..20: mol_type = other DNA
ccgagcgagcccgccgccgc

SEQ ID NO: 25 - DNA, 20 bp, synthetic construct
  source 1..20: mol_type = other DNA
cctcggcgggtgtgatcgag

SEQ ID NO: 26 - DNA, 20 bp, synthetic construct
  source 1..20: mol_type = other DNA
ggcccgcgctcactgcgcgc

SEQ ID NO: 27 - DNA, 20 bp, synthetic construct
  source 1..20: mol_type = other DNA
gcgggagcgccgcgctcggg

SEQ ID NO: 28 - DNA, 20 bp, synthetic construct
  source 1..20: mol_type = other DNA
cggaggcggcggcgactgag

SEQ ID NO: 29 - DNA, 20 bp, synthetic construct
  source 1..20: mol_type = other DNA
ctcgctcgggccgtagctga

SEQ ID NO: 30 - DNA, 20 bp, synthetic construct
  source 1..20: mol_type = other DNA
cccagggagcggggccgctt

SEQ ID NO: 31 - DNA, 20 bp, synthetic construct
  source 1..20: mol_type = other DNA
cggcggcggcgcggagaaca

SEQ ID NO: 32 - DNA, 20 bp, synthetic construct
  source 1..20: mol_type = other DNA
tcggcctccctcacccgcgg

SEQ ID NO: 33 - DNA, 20 bp, synthetic construct
  source 1..20: mol_type = other DNA
tggctcgctggctgcacggc

SEQ ID NO: 34 - DNA, 20 bp, synthetic construct
  source 1..20: mol_type = other DNA
ccgaagcggccccgctccct

SEQ ID NO: 35 - DNA, 20 bp, synthetic construct
  source 1..20: mol_type = other DNA
cgcccgccggccatgtcccc

SEQ ID NO: 36 - DNA, 20 bp, synthetic construct
  source 1..20: mol_type = other DNA
gcggaggcggcggcgactga

SEQ ID NO: 37 - DNA, 20 bp, synthetic construct
  source 1..20: mol_type = other DNA
tcgggccgtagctgaaggcg

SEQ ID NO: 38 - DNA, 20 bp, synthetic construct
  source 1..20: mol_type = other DNA
ctccaaacccaacatggcgg

SEQ ID NO: 39 - DNA, 20 bp, synthetic construct
  source 1..20: mol_type = other DNA
cttgccgttcgcccgcccca

SEQ ID NO: 40 - DNA, 20 bp, synthetic construct
  source 1..20: mol_type = other DNA
ccgccgccgccgcccgagcg

SEQ ID NO: 41 - DNA, 20 bp, synthetic construct
  source 1..20: mol_type = other DNA
tgcacggcgggccgggaagg

SEQ ID NO: 42 - DNA, 20 bp, synthetic construct
  source 1..20: mol_type = other DNA
ggagcgccgcgctcgggcgg

SEQ ID NO: 43 - DNA, 20 bp, synthetic construct
  source 1..20: mol_type = other DNA
ggccgcgggagcgccgcgct

SEQ ID NO: 44 - DNA, 20 bp, synthetic construct
  source 1..20: mol_type = other DNA
cggcggccgggggacatggc

SEQ ID NO: 45 - DNA, 20 bp, synthetic construct
  source 1..20: mol_type = other DNA
ggcccggccacagcctgcag

SEQ ID NO: 46 - DNA, 20 bp, synthetic construct
  source 1..20: mol_type = other DNA
tccgaagcggccccgctccc

SEQ ID NO: 47 - DNA, 20 bp, synthetic construct
  source 1..20: mol_type = other DNA
gcggagaacaagggggccct

SEQ ID NO: 48 - DNA, 20 bp, synthetic construct
  source 1..20: mol_type = other DNA
gccgccgccgccgccatgtt

SEQ ID NO: 49 - DNA, 20 bp, synthetic construct
  source 1..20: mol_type = other DNA
cagctccaaacccaacatgg

SEQ ID NO: 50 - DNA, 20 bp, synthetic construct
  source 1..20: mol_type = other DNA
agaacaagggggccctgggg

SEQ ID NO: 51 - DNA, 20 bp, synthetic construct
  source 1..20: mol_type = other DNA
gggcgctaggcgatgaggcg

SEQ ID NO: 52 - DNA, 20 bp, synthetic construct
  source 1..20: mol_type = other DNA
gggcccgcgctcactgcgcg

SEQ ID NO: 53 - DNA, 20 bp, synthetic construct
  source 1..20: mol_type = other DNA
acatggccggcgggcggagg

SEQ ID NO: 54 - DNA, 20 bp, synthetic construct
  source 1..20: mol_type = other DNA
tcgctggctcgctggctgca

SEQ ID NO: 55 - DNA, 20 bp, synthetic construct
  source 1..20: mol_type = other DNA
tcgccgccgcctccgcccgc

SEQ ID NO: 56 - DNA, 20 bp, synthetic construct
  source 1..20: mol_type = other DNA
gcccgagcgcggcgctcccg

SEQ ID NO: 57 - DNA, 20 bp, synthetic construct
  source 1..20: mol_type = other DNA
ggccccgcgcgcagtgagcg

SEQ ID NO: 58 - DNA, 20 bp, synthetic construct
  source 1..20: mol_type = other DNA
ctgcagctccaaacccaaca

SEQ ID NO: 59 - DNA, 20 bp, synthetic construct
  source 1..20: mol_type = other DNA
ggccgggggacatggccggc

SEQ ID NO: 60 - DNA, 20 bp, synthetic construct
  source 1..20: mol_type = other DNA
cggcgactgaggggggcgct

SEQ ID NO: 61 - DNA, 20 bp, synthetic construct
  source 1..20: mol_type = other DNA
caggctgtggccgggcccgg

SEQ ID NO: 62 - DNA, 20 bp, synthetic construct
  source 1..20: mol_type = other DNA
gcctccctcacccgcggcgg

SEQ ID NO: 63 - DNA, 20 bp, synthetic construct
  source 1..20: mol_type = other DNA
gaggcggcggcgactgaggg

SEQ ID NO: 64 - DNA, 20 bp, synthetic construct
  source 1..20: mol_type = other DNA
gcccacgagaggcagcgcca

SEQ ID NO: 65 - DNA, 20 bp, synthetic construct
  source 1..20: mol_type = other DNA
gcgagcaagcaagcaagcac

SEQ ID NO: 66 - DNA, 20 bp, synthetic construct
  source 1..20: mol_type = other DNA
ggaggcggcggcgactgagg

SEQ ID NO: 67 - DNA, 20 bp, synthetic construct
  source 1..20: mol_type = other DNA
gggacatggccggcgggcgg

SEQ ID NO: 68 - DNA, 20 bp, synthetic construct
  source 1..20: mol_type = other DNA
cacgagaggcagcgccatgg

SEQ ID NO: 69 - DNA, 20 bp, synthetic construct
  source 1..20: mol_type = other DNA
cgccgccgccatgttgggtt

SEQ ID NO: 70 - DNA, 20 bp, synthetic construct
  source 1..20: mol_type = other DNA
ccgtagctgaaggcgcggcc

SEQ ID NO: 71 - DNA, 20 bp, synthetic construct
  source 1..20: mol_type = other DNA
gcccgcgctcactgcgcgcg

SEQ ID NO: 72 - DNA, 20 bp, synthetic construct
  source 1..20: mol_type = other DNA
gagcggagcccgccccgccc

SEQ ID NO: 73 - DNA, 20 bp, synthetic construct
  source 1..20: mol_type = other DNA
cggagaacaagggggccctg

SEQ ID NO: 74 - DNA, 20 bp, synthetic construct
  source 1..20: mol_type = other DNA
cctctcgtgggctccgctgc

SEQ ID NO: 75 - DNA, 20 bp, synthetic construct
  source 1..20: mol_type = other DNA
ttgcttgcttgctcgctcgc

SEQ ID NO: 76 - DNA, 20 bp, synthetic construct
  source 1..20: mol_type = other DNA
cggccgggggacatggccgg

SEQ ID NO: 77 - DNA, 20 bp, synthetic construct
  source 1..20: mol_type = other DNA
gccccgctccctgggccccg

SEQ ID NO: 78 - DNA, 20 bp, synthetic construct
  source 1..20: mol_type = other DNA
caaacccaacatggcggcgg

SEQ ID NO: 79 - DNA, 20 bp, synthetic construct
  source 1..20: mol_type = other DNA
ggcggggcgggctccgctct

SEQ ID NO: 80 - DNA, 20 bp, synthetic construct
  source 1..20: mol_type = other DNA
cgagcgagcccgccgccgcc

SEQ ID NO: 81 - DNA, 20 bp, synthetic construct
  source 1..20: mol_type = other DNA
ctccccgccagccgccttcc

SEQ ID NO: 82 - DNA, 20 bp, synthetic construct
  source 1..20: mol_type = other DNA
tgttgggtttggagctgcag

SEQ ID NO: 83 - DNA, 20 bp, synthetic construct
  source 1..20: mol_type = other DNA
ctcactgcgcgcggggccgc

SEQ ID NO: 84 - DNA, 20 bp, synthetic construct
  source 1..20: mol_type = other DNA
cggcgggccgggaaggcggc

SEQ ID NO: 85 - DNA, 20 bp, synthetic construct
  source 1..20: mol_type = other DNA
cgggtgagggaggccgagag

SEQ ID NO: 86 - DNA, 20 bp, synthetic construct
  source 1..20: mol_type = other DNA
cgggccgggaaggcggctgg

SEQ ID NO: 87 - DNA, 20 bp, synthetic construct
  source 1..20: mol_type = other DNA
gggccgggaaggcggctggc

SEQ ID NO: 88 - DNA, 20 bp, synthetic construct
  source 1..20: mol_type = other DNA
cgcggagaacaagggggccc

SEQ ID NO: 89 - DNA, 20 bp, synthetic construct
  source 1..20: mol_type = other DNA
gccgtagctgaaggcgcggc

SEQ ID NO: 90 - DNA, 20 bp, synthetic construct
  source 1..20: mol_type = other DNA
gccgccgccgccgcgggtga

SEQ ID NO: 91 - DNA, 20 bp, synthetic construct
  source 1..20: mol_type = other DNA
ccggcggcggcgggctcgct

SEQ ID NO: 92 - DNA, 20 bp, synthetic construct
  source 1..20: mol_type = other DNA
ctgaaggcgcggccggggtc

SEQ ID NO: 93 - DNA, 20 bp, synthetic construct
  source 1..20: mol_type = other DNA
ggctgcacggcgggccggga

SEQ ID NO: 94 - DNA, 20 bp, synthetic construct
  source 1..20: mol_type = other DNA
gccgcgggagcgccgcgctc

SEQ ID NO: 95 - DNA, 20 bp, synthetic construct
  source 1..20: mol_type = other DNA
gctcactgcgcgcggggccg

SEQ ID NO: 96 - DNA, 20 bp, synthetic construct
  source 1..20: mol_type = other DNA
ggggccctggggcgggcgaa

SEQ ID NO: 97 - DNA, 20 bp, synthetic construct
  source 1..20: mol_type = other DNA
gtgggctccgctgcaggctg

SEQ ID NO: 98 - DNA, 20 bp, synthetic construct
  source 1..20: mol_type = other DNA
gcggagcccgccccgccccg

SEQ ID NO: 99 - DNA, 20 bp, synthetic construct
  source 1..20: mol_type = other DNA
tggccggcgggcggaggcgg

SEQ ID NO: 100 - DNA, 20 bp, synthetic construct
  source 1..20: mol_type = other DNA
cgggggacatggccggcggg

SEQ ID NO: 101 - DNA, 20 bp, synthetic construct
  source 1..20: mol_type = other DNA
cgccatggcgctgcctctcg

SEQ ID NO: 102 - DNA, 20 bp, synthetic construct
  source 1..20: mol_type = other DNA
gaacaagggggccctggggc

SEQ ID NO: 103 - DNA, 20 bp, synthetic construct
  source 1..20: mol_type = other DNA
gctccgctgcaggctgtggc

SEQ ID NO: 104 - DNA, 20 bp, synthetic construct
  source 1..20: mol_type = other DNA
ttgctcgctcgctggctcgc

SEQ ID NO: 105 - DNA, 20 bp, synthetic construct
  source 1..20: mol_type = other DNA
cgtagctgaaggcgcggccg

SEQ ID NO: 106 - DNA, 20 bp, synthetic construct
  source 1..20: mol_type = other DNA
gctgtggccgggcccggcgg

SEQ ID NO: 107 - DNA, 20 bp, synthetic construct
  source 1..20: mol_type = other DNA
tcgctggctgcacggcgggc

SEQ ID NO: 108 - DNA, 20 bp, synthetic construct
  source 1..20: mol_type = other DNA
gcggcggcggccgggggaca

SEQ ID NO: 109 - DNA, 20 bp, synthetic construct
  source 1..20: mol_type = other DNA
ggccgggaaggcggctggcg

SEQ ID NO: 110 - DNA, 20 bp, synthetic construct
  source 1..20: mol_type = other DNA
gccgccgccgcgggtgaggg

SEQ ID NO: 111 - DNA, 20 bp, synthetic construct
  source 1..20: mol_type = other DNA
tccctcacccgcggcggcgg

SEQ ID NO: 112 - DNA, 20 bp, synthetic construct
  source 1..20: mol_type = other DNA
acccaacatggcggcggcgg

SEQ ID NO: 113 - DNA, 20 bp, synthetic construct
  source 1..20: mol_type = other DNA
agcggggccgcttcggagcc

SEQ ID NO: 114 - DNA, 20 bp, synthetic construct
  source 1..20: mol_type = other DNA
ccgcgctcgggcggcggcgg

SEQ ID NO: 115 - DNA, 20 bp, synthetic construct
  source 1..20: mol_type = other DNA
agcggagcccgccccgcccc

SEQ ID NO: 116 - DNA, 20 bp, synthetic construct
  source 1..20: mol_type = other DNA
ctccgctgcaggctgtggcc

SEQ ID NO: 117 - RNA, 20 nt, synthetic construct
  source 1..20: mol_type = other RNA
cgctggctgcacggcgggcc

SEQ ID NO: 118 - DNA, 20 bp, synthetic construct
  source 1..20: mol_type = other DNA
gcggctggcggggagaggcc

SEQ ID NO: 119 - DNA, 20 bp, synthetic construct
  source 1..20: mol_type = other DNA
tggccgggcccggcggcggc

SEQ ID NO: 120 - DNA, 20 bp, synthetic construct
  source 1..20: mol_type = other DNA
gccccggggcccagggagcg

SEQ ID NO: 121 - DNA, 20 bp, synthetic construct
  source 1..20: mol_type = other DNA
ctgcaggctgtggccgggcc

SEQ ID NO: 122 - DNA, 20 bp, synthetic construct
  source 1..20: mol_type = other DNA
cgccgccgccgccgccatgt

SEQ ID NO: 123 - DNA, 20 bp, synthetic construct
  source 1..20: mol_type = other DNA
cgctcgggcggcggcggcgg

SEQ ID NO: 124 - DNA, 20 bp, synthetic construct
  source 1..20: mol_type = other DNA
ccgctccctgggccccgggg

SEQ ID NO: 125 - DNA, 20 bp, synthetic construct
  source 1..20: mol_type = other DNA
ctcacccgcggcggcggcgg

SEQ ID NO: 126 - DNA, 20 bp, synthetic construct
  source 1..20: mol_type = other DNA
ggcggaggcggcggcgactg

SEQ ID NO: 127 - DNA, 20 bp, synthetic construct
  source 1..20: mol_type = other DNA
gcgccgcgctcgggcggcgg

SEQ ID NO: 128 - DNA, 20 bp, synthetic construct
  source 1..20: mol_type = other DNA
gcggcggcggcggcggccgg

SEQ ID NO: 129 - DNA, 20 bp, synthetic construct
  source 1..20: mol_type = other DNA
ggaaggcggctggcggggag

SEQ ID NO: 130 - DNA, 20 bp, synthetic construct
  source 1..20: mol_type = other DNA
ccgccccggggcccagggag

SEQ ID NO: 131 - DNA, 20 bp, synthetic construct
  source 1..20: mol_type = other DNA
gtggccgggcccggcggcgg

SEQ ID NO: 132 - DNA, 20 bp, synthetic construct
  source 1..20: mol_type = other DNA
cccgccccgccccggggccc

SEQ ID NO: 133 - DNA, 20 bp, synthetic construct
  source 1..20: mol_type = other DNA
ccgccccgccccggggccca

SEQ ID NO: 134 - DNA, 20 bp, synthetic construct
  source 1..20: mol_type = other DNA
ggccccgctccctgggcccc

SEQ ID NO: 135 - DNA, 20 bp, synthetic construct
  source 1..20: mol_type = other DNA
ggcggctggcggggagaggc

SEQ ID NO: 136 - DNA, 20 bp, synthetic construct
  source 1..20: mol_type = other DNA
gctccctgggccccggggcg

SEQ ID NO: 137 - DNA, 20 bp, synthetic construct
  source 1..20: mol_type = other DNA
cggagccgccgccgccgccg

SEQ ID NO: 138 - DNA, 20 bp, synthetic construct
  source 1..20: mol_type = other DNA
ccctgggccccggggcgggg

SEQ ID NO: 139 - DNA, 20 bp, synthetic construct
  source 1..20: mol_type = other DNA
cgccccggggcccagggagc

SEQ ID NO: 140 - DNA, 20 bp, synthetic construct
  source 1..20: mol_type = other DNA
cggccccgctccctgggccc

SEQ ID NO: 141 - DNA, 20 bp, synthetic construct
  source 1..20: mol_type = other DNA
cctgggccccggggcggggc

SEQ ID NO: 142 - DNA, 20 bp, synthetic construct
  source 1..20: mol_type = other DNA
gagcccgccgccgccgggcc

SEQ ID NO: 143 - DNA, 20 bp, synthetic construct
  source 1..20: mol_type = other DNA
cgctccctgggccccggggc

SEQ ID NO: 144 - DNA, 20 bp, synthetic construct
  source 1..20: mol_type = other DNA
cgccgccgccgccgcgggtg

SEQ ID NO: 145 - DNA, 20 bp, synthetic construct
  source 1..20: mol_type = other DNA
cacttgactggaatccacca

SEQ ID NO: 146 - DNA, 20 bp, synthetic construct
  source 1..20: mol_type = other DNA
acacttgactggaatccacc

SEQ ID NO: 147 - DNA, 20 bp, synthetic construct
  source 1..20: mol_type = other DNA
accatagactataagaagaa

SEQ ID NO: 148 - DNA, 20 bp, synthetic construct
  source 1..20: mol_type = other DNA
tccattcttcttatagtcta

SEQ ID NO: 149 - DNA, 20 bp, synthetic construct
  source 1..20: mol_type = other DNA
cagaaatgtagacacttgac

SEQ ID NO: 150 - DNA, 20 bp, synthetic construct
  source 1..20: mol_type = other DNA
aagacagtaatagttcttct

SEQ ID NO: 151 - DNA, 20 bp, synthetic construct
  source 1..20: mol_type = other DNA
aaagacagtaatagttcttc

SEQ ID NO: 152 - DNA, 20 bp, synthetic construct
  source 1..20: mol_type = other DNA
agttcttctgggtctttcaa

SEQ ID NO: 153 - DNA, 20 bp, synthetic construct
  source 1..20: mol_type = other DNA
ggactttgaaaatcaagata

SEQ ID NO: 154 - DNA, 20 bp, synthetic construct
  source 1..20: mol_type = other DNA
agagagacagatgctccaat

SEQ ID NO: 155 - DNA, 20 bp, synthetic construct
  source 1..20: mol_type = other DNA
agacagatgctccaattgga

SEQ ID NO: 156 - DNA, 20 bp, synthetic construct
  source 1..20: mol_type = other DNA
cctgggtagagtcaattgtt

SEQ ID NO: 157 - DNA, 20 bp, synthetic construct
  source 1..20: mol_type = other DNA
caggctctgttccttccaat

SEQ ID NO: 158 - DNA, 20 bp, synthetic construct
  source 1..20: mol_type = other DNA
aattggaaggaacagagcct

SEQ ID NO: 159 - DNA, 20 bp, synthetic construct
  source 1..20: mol_type = other DNA
ccaaacaattgactctaccc

SEQ ID NO: 160 - DNA, 20 bp, synthetic construct
  source 1..20: mol_type = other DNA
caattggaaggaacagagcc

SEQ ID NO: 161 - DNA, 20 bp, synthetic construct
  source 1..20: mol_type = other DNA
agcagggtcttgttaaatac

SEQ ID NO: 162 - DNA, 20 bp, synthetic construct
  source 1..20: mol_type = other DNA
cttgttaaatactggcacat

SEQ ID NO: 163 - DNA, 20 bp, synthetic construct
  source 1..20: mol_type = other DNA
ttgttaaatactggcacatc

SEQ ID NO: 164 - DNA, 20 bp, synthetic construct
  source 1..20: mol_type = other DNA
ttaaatactggcacatcggg

SEQ ID NO: 165 - DNA, 20 bp, synthetic construct
  source 1..20: mol_type = other DNA
ggccagtgagaacccagatg

SEQ ID NO: 166 - DNA, 20 bp, synthetic construct
  source 1..20: mol_type = other DNA
gaaacgtccacagcaaccaa

SEQ ID NO: 167 - DNA, 20 bp, synthetic construct
  source 1..20: mol_type = other DNA
tctgggttctcactggccat

SEQ ID NO: 168 - DNA, 20 bp, synthetic construct
  source 1..20: mol_type = other DNA
gtcctcatctgggttctcac

SEQ ID NO: 169 - DNA, 20 bp, synthetic construct
  source 1..20: mol_type = other DNA
cactggccattggcttctca

SEQ ID NO: 170 - DNA, 20 bp, synthetic construct
  source 1..20: mol_type = other DNA
tgtcatgctcgtcctcatct

SEQ ID NO: 171 - DNA, 20 bp, synthetic construct
  source 1..20: mol_type = other DNA
ctgtcatgctcgtcctcatc

SEQ ID NO: 172 - DNA, 20 bp, synthetic construct
  source 1..20: mol_type = other DNA
aggcaggagaccttgaggct

SEQ ID NO: 173 - DNA, 20 bp, synthetic construct
  source 1..20: mol_type = other DNA
caggcggacaaaggcgatca

SEQ ID NO: 174 - DNA, 20 bp, synthetic construct
  source 1..20: mol_type = other DNA
aggcgatcatggcgacacag

SEQ ID NO: 175 - DNA, 20 bp, synthetic construct
  source 1..20: mol_type = other DNA
gaggctcggcaggcggacaa

SEQ ID NO: 176 - DNA, 20 bp, synthetic construct
  source 1..20: mol_type = other DNA
catggcgacacagaggccca

SEQ ID NO: 177 - DNA, 20 bp, synthetic construct
  source 1..20: mol_type = other DNA
aggagaccttgaggctcggc

SEQ ID NO: 178 - DNA, 20 bp, synthetic construct
  source 1..20: mol_type = other DNA
tgtccgcctgccgagcctca

SEQ ID NO: 179 - DNA, 20 bp, synthetic construct
  source 1..20: mol_type = other DNA
tgagaagccctgagagaagc

SEQ ID NO: 180 - DNA, 20 bp, synthetic construct
  source 1..20: mol_type = other DNA
gaagcaggcaggagaccttg

SEQ ID NO: 181 - DNA, 20 bp, synthetic construct
  source 1..20: mol_type = other DNA
agaccttgaggctcggcagg

SEQ ID NO: 182 - DNA, 20 bp, synthetic construct
  source 1..20: mol_type = other DNA
aagccctgagagaagcaggc

SEQ ID NO: 183 - DNA, 20 bp, synthetic construct
  source 1..20: mol_type = other DNA
gtctcctgcctgcttctctc

SEQ ID NO: 184 - DNA, 20 bp, synthetic construct
  source 1..20: mol_type = other DNA
atccccttgacgttctatcc

SEQ ID NO: 185 - DNA, 20 bp, synthetic construct
  source 1..20: mol_type = other DNA
ggaacatcacgcccaacatt

SEQ ID NO: 186 - DNA, 20 bp, synthetic construct
  source 1..20: mol_type = other DNA
tccacctggggcccaatgtt

SEQ ID NO: 187 - DNA, 20 bp, synthetic construct
  source 1..20: mol_type = other DNA
tctatcccggaagctccacc

SEQ ID NO: 188 - DNA, 20 bp, synthetic construct
  source 1..20: mol_type = other DNA
gcttccgggatagaacgtca

SEQ ID NO: 189 - DNA, 20 bp, synthetic construct
  source 1..20: mol_type = other DNA
acgtcaaggggattgtcagc

SEQ ID NO: 190 - DNA, 20 bp, synthetic construct
  source 1..20: mol_type = other DNA
aggaacatcacgcccaacat

SEQ ID NO: 191 - DNA, 20 bp, synthetic construct
  source 1..20: mol_type = other DNA
tatcccggaagctccacctg

SEQ ID NO: 192 - DNA, 20 bp, synthetic construct
  source 1..20: mol_type = other DNA
ggtgaaggtggccactcagc

SEQ ID NO: 193 - DNA, 20 bp, synthetic construct
  source 1..20: mol_type = other DNA
cttccgggatagaacgtcaa

SEQ ID NO: 194 - DNA, 20 bp, synthetic construct
  source 1..20: mol_type = other DNA
ctatcccggaagctccacct

SEQ ID NO: 195 - DNA, 20 bp, synthetic construct
  source 1..20: mol_type = other DNA
ttccgggatagaacgtcaag

SEQ ID NO: 196 - DNA, 20 bp, synthetic construct
  source 1..20: mol_type = other DNA
gggattgtcagccggctgag

SEQ ID NO: 197 - DNA, 20 bp, synthetic construct
  source 1..20: mol_type = other DNA
gacgttgctattgaagatgt

SEQ ID NO: 198 - DNA, 20 bp, synthetic construct
  source 1..20: mol_type = other DNA
caatagcaacgtcatggtga

SEQ ID NO: 199 - DNA, 20 bp, synthetic construct
  source 1..20: mol_type = other DNA
tagcaacgtcatggtgaagg

SEQ ID NO: 200 - DNA, 20 bp, synthetic construct
  source 1..20: mol_type = other DNA
catcttcaatagcaacgtca

SEQ ID NO: 201 - DNA, 20 bp, synthetic construct
  source 1..20: mol_type = other DNA
gcccaacattgggccccagg

SEQ ID NO: 202 - DNA, 21 bp, synthetic construct
  source 1..21: mol_type = other DNA
ctccacctgggsgcccaatgt

SEQ ID NO: 203 - DNA, 20 bp, synthetic construct
  source 1..20: mol_type = other DNA
gggccccaggtggagcttcc

SEQ ID NO: 204 - DNA, 20 bp, synthetic construct
  source 1..20: mol_type = other DNA
cacgcccaacattgggcccc

SEQ ID NO: 205 - DNA, 20 bp, synthetic construct
  source 1..20: mol_type = other DNA
tttccaggcagagacaggcg

SEQ ID NO: 206 - DNA, 20 bp, synthetic construct
  source 1..20: mol_type = other DNA
tgggccccaggtggagcttc

SEQ ID NO: 207 - DNA, 20 bp, synthetic construct
  source 1..20: mol_type = other DNA
cctgtctctgcctggaaaac

SEQ ID NO: 208 - DNA, 20 bp, synthetic construct
  source 1..20: mol_type = other DNA
gttcctcgcctgtctctgcc

SEQ ID NO: 209 - DNA, 20 bp, synthetic construct
  source 1..20: mol_type = other DNA
acaaagcatagtaggagacc

SEQ ID NO: 210 - DNA, 20 bp, synthetic construct
  source 1..20: mol_type = other DNA
gatgagggtgcagtgaaagt

SEQ ID NO: 211 - DNA, 20 bp, synthetic construct
  source 1..20: mol_type = other DNA
agcgaaggacaaagcatagt

SEQ ID NO: 212 - DNA, 20 bp, synthetic construct
  source 1..20: mol_type = other DNA
gatgtctccgatgcccaaca

SEQ ID NO: 213 - DNA, 20 bp, synthetic construct
  source 1..20: mol_type = other DNA
actacaaaaagcaagccagt

SEQ ID NO: 214 - DNA, 20 bp, synthetic construct
  source 1..20: mol_type = other DNA
ctggacctgccaacatctcc

SEQ ID NO: 215 - DNA, 20 bp, synthetic construct
  source 1..20: mol_type = other DNA
ggcagccacttctccatgtt

SEQ ID NO: 216 - DNA, 20 bp, synthetic construct
  source 1..20: mol_type = other DNA
ggccccacaggagtccccac

SEQ ID NO: 217 - DNA, 20 bp, synthetic construct
  source 1..20: mol_type = other DNA
ctgcatgcgcccggagatgt

SEQ ID NO: 218 - DNA, 20 bp, synthetic construct
  source 1..20: mol_type = other DNA
catctccgggcgcatgcaga

SEQ ID NO: 219 - DNA, 20 bp, synthetic construct
  source 1..20: mol_type = other DNA
tactttcactgcaccctcat

SEQ ID NO: 220 - DNA, 20 bp, synthetic construct
  source 1..20: mol_type = other DNA
atcggagacatcgttatgcc

SEQ ID NO: 221 - DNA, 20 bp, synthetic construct
  source 1..20: mol_type = other DNA
cgatgcccaacatggagaag

SEQ ID NO: 222 - DNA, 20 bp, synthetic construct
  source 1..20: mol_type = other DNA
aagccagtggggactcctgt

SEQ ID NO: 223 - DNA, 20 bp, synthetic construct
  source 1..20: mol_type = other DNA
ctacaaaaagcaagccagtg

SEQ ID NO: 224 - DNA, 20 bp, synthetic construct
  source 1..20: mol_type = other DNA
agccagtggggactcctgtg

SEQ ID NO: 225 - DNA, 20 bp, synthetic construct
  source 1..20: mol_type = other DNA
atgcgcccggagatgttggc

SEQ ID NO: 226 - DNA, 20 bp, synthetic construct
  source 1..20: mol_type = other DNA
tggcagccacttctccatgt

SEQ ID NO: 227 - DNA, 20 bp, synthetic construct
  source 1..20: mol_type = other DNA
cctggacctgccaacatctc

SEQ ID NO: 228 - DNA, 20 bp, synthetic construct
  source 1..20: mol_type = other DNA
aactacaaaaagcaagccag

SEQ ID NO: 229 - DNA, 20 bp, synthetic construct
  source 1..20: mol_type = other DNA
ggagaccttctgcatgcgcc

SEQ ID NO: 230 - DNA, 20 bp, synthetic construct
  source 1..20: mol_type = other DNA
caagccagtggggactcctg

SEQ ID NO: 231 - DNA, 20 bp, synthetic construct
  source 1..20: mol_type = other DNA
ggagatgttggcaggtccag

SEQ ID NO: 232 - DNA, 20 bp, synthetic construct
  source 1..20: mol_type = other DNA
cacttctccatgttgggcat

SEQ ID NO: 233 - DNA, 20 bp, synthetic construct
  source 1..20: mol_type = other DNA
cggagatgttggcaggtcca

SEQ ID NO: 234 - DNA, 20 bp, synthetic construct
  source 1..20: mol_type = other DNA
ggcaggtccaggggccccac

SEQ ID NO: 235 - DNA, 20 bp, synthetic construct
  source 1..20: mol_type = other DNA
ccggagatgttggcaggtcc

SEQ ID NO: 236 - DNA, 20 bp, synthetic construct
  source 1..20: mol_type = other DNA
ggggactcctgtggggcccc

SEQ ID NO: 237 - DNA, 20 bp, synthetic construct
  source 1..20: mol_type = other DNA
acaaagcatagtaggagacc

SEQ ID NO: 238 - DNA, 20 bp, synthetic construct
  source 1..20: mol_type = other DNA
aaataggccatcgtgaggag

SEQ ID NO: 239 - DNA, 20 bp, synthetic construct
  source 1..20: mol_type = other DNA
aggagtggcaataaagtaaa

SEQ ID NO: 240 - DNA, 20 bp, synthetic construct
  source 1..20: mol_type = other DNA
tttattgccactcctcacga

SEQ ID NO: 241 - DNA, 20 bp, synthetic construct
  source 1..20: mol_type = other DNA
tggcaccaaatagagaaggg

SEQ ID NO: 242 - DNA, 20 bp, synthetic construct
  source 1..20: mol_type = other DNA
aaatggcaccaaatagagaa

SEQ ID NO: 243 - DNA, 20 bp, synthetic construct
  source 1..20: mol_type = other DNA
ggcaccaaatagagaagggc

SEQ ID NO: 244 - DNA, 20 bp, synthetic construct
  source 1..20: mol_type = other DNA
taaatggcaccaaatagaga

SEQ ID NO: 245 - DNA, 20 bp, synthetic construct
  source 1..20: mol_type = other DNA
ccagcccgcccttctctatt

SEQ ID NO: 246 - DNA, 20 bp, synthetic construct
  source 1..20: mol_type = other DNA
ccaaatagagaagggcgggc

SEQ ID NO: 247 - DNA, 20 bp, synthetic construct
  source 1..20: mol_type = other DNA
atagagaagggcgggctggg

SEQ ID NO: 248 - DNA, 20 bp, synthetic construct
  source 1..20: mol_type = other DNA
caaatagagaagggcgggct

SEQ ID NO: 249 - DNA, 20 bp, synthetic construct
  source 1..20: mol_type = other DNA
gaagggcgggctgggcggcc

SEQ ID NO: 250 - DNA, 20 bp, synthetic construct
  source 1..20: mol_type = other DNA
aaggctcagaccacatccgc

SEQ ID NO: 251 - DNA, 20 bp, synthetic construct
  source 1..20: mol_type = other DNA
gctcagaccacatccgccgg

SEQ ID NO: 252 - DNA, 20 bp, synthetic construct
  source 1..20: mol_type = other DNA
gtccagcagctcccgattcc

SEQ ID NO: 253 - DNA, 20 bp, synthetic construct
  source 1..20: mol_type = other DNA
ctgctggacttggagtggaa

SEQ ID NO: 254 - DNA, 20 bp, synthetic construct
  source 1..20: mol_type = other DNA
ttccaggaatcgggagctgc

SEQ ID NO: 255 - DNA, 20 bp, synthetic construct
  source 1..20: mol_type = other DNA
gggagctgctggacttggag

SEQ ID NO: 256 - DNA, 20 bp, synthetic construct
  source 1..20: mol_type = other DNA
gaatcgggagctgctggact

SEQ ID NO: 257 - DNA, 20 bp, synthetic construct
  source 1..20: mol_type = other DNA
caggaggaggattcggaacc

SEQ ID NO: 258 - DNA, 20 bp, synthetic construct
  source 1..20: mol_type = other DNA
tcgaccagcttgacatcaca

SEQ ID NO: 259 - DNA, 20 bp, synthetic construct
  source 1..20: mol_type = other DNA
aatctgctcatgacgctgcg

SEQ ID NO: 260 - DNA, 20 bp, synthetic construct
  source 1..20: mol_type = other DNA
tggatatctgtgggacaaga

SEQ ID NO: 261 - DNA, 20 bp, synthetic construct
  source 1..20: mol_type = other DNA
ttcttatagtctatggtagt

SEQ ID NO: 262 - DNA, 20 bp, synthetic construct
  source 1..20: mol_type = other DNA
cctggtggattccagtcaag

SEQ ID NO: 263 - DNA, 20 bp, synthetic construct
  source 1..20: mol_type = other DNA
ctgatttccattcttcttat

SEQ ID NO: 264 - DNA, 20 bp, synthetic construct
  source 1..20: mol_type = other DNA
tgatttccattcttcttata

SEQ ID NO: 265 - DNA, 20 bp, synthetic construct
  source 1..20: mol_type = other DNA
ccattcttcttatagtctat

SEQ ID NO: 266 - DNA, 20 bp, synthetic construct
  source 1..20: mol_type = other DNA
cattcttcttatagtctatg

SEQ ID NO: 267 - DNA, 20 bp, synthetic construct
  source 1..20: mol_type = other DNA
cctgaaactaccatagacta

SEQ ID NO: 268 - DNA, 20 bp, synthetic construct
  source 1..20: mol_type = other DNA
ttatagtctatggtagtttc

SEQ ID NO: 269 - DNA, 20 bp, synthetic construct
  source 1..20: mol_type = other DNA
tgggtctttcaatggcaaca

SEQ ID NO: 270 - DNA, 20 bp, synthetic construct
  source 1..20: mol_type = other DNA
caatggcaacagcaccaata

SEQ ID NO: 271 - DNA, 20 bp, synthetic construct
  source 1..20: mol_type = other DNA
gaaaatcaagataaggagaa

SEQ ID NO: 272 - DNA, 20 bp, synthetic construct
  source 1..20: mol_type = other DNA
aaaatcaagataaggagaaa

SEQ ID NO: 273 - DNA, 20 bp, synthetic construct
  source 1..20: mol_type = other DNA
ttctgggtctttcaatggca

SEQ ID NO: 274 - DNA, 20 bp, synthetic construct
  source 1..20: mol_type = other DNA
aatggcaacagcaccaataa

SEQ ID NO: 275 - DNA, 20 bp, synthetic construct
  source 1..20: mol_type = other DNA
ctgtctttctccttatcttg

SEQ ID NO: 276 - DNA, 20 bp, synthetic construct
  source 1..20: mol_type = other DNA
aaagacccagaagaactatt

SEQ ID NO: 277 - DNA, 20 bp, synthetic construct
  source 1..20: mol_type = other DNA
ccattgaaagacccagaaga

SEQ ID NO: 278 - DNA, 20 bp, synthetic construct
  source 1..20: mol_type = other DNA
gtgctgttgccattgaaaga

SEQ ID NO: 279 - DNA, 20 bp, synthetic construct
  source 1..20: mol_type = other DNA
ttggtgctgttgccattgaa

SEQ ID NO: 280 - DNA, 20 bp, synthetic construct
  source 1..20: mol_type = other DNA
ctccttatcttgattttcaa

SEQ ID NO: 281 - DNA, 20 bp, synthetic construct
  source 1..20: mol_type = other DNA
caggcatccaaacaattgac

SEQ ID NO: 282 - DNA, 20 bp, synthetic construct
  source 1..20: mol_type = other DNA
caattggagcatctgtctct

SEQ ID NO: 283 - DNA, 20 bp, synthetic construct
  source 1..20: mol_type = other DNA
tagtaatgttcttcttcttt

SEQ ID NO: 284 - DNA, 20 bp, synthetic construct
  source 1..20: mol_type = other DNA
ttctttgactcagttcaagt

SEQ ID NO: 285 - DNA, 20 bp, synthetic construct
  source 1..20: mol_type = other DNA
tttgactcagttcaagtagt

SEQ ID NO: 286 - DNA, 20 bp, synthetic construct
  source 1..20: mol_type = other DNA
gactcagttcaagtagtttt

SEQ ID NO: 287 - DNA, 20 bp, synthetic construct
  source 1..20: mol_type = other DNA
cttccaattggagcatctgt

SEQ ID NO: 288 - DNA, 20 bp, synthetic construct
  source 1..20: mol_type = other DNA
ttcttctttgactcagttca

SEQ ID NO: 289 - DNA, 20 bp, synthetic construct
  source 1..20: mol_type = other DNA
aagtagtttttacaatatgt

SEQ ID NO: 290 - DNA, 20 bp, synthetic construct
  source 1..20: mol_type = other DNA
tgaggtgagcagggtcttgt

SEQ ID NO: 291 - DNA, 20 bp, synthetic construct
  source 1..20: mol_type = other DNA
tgcttttcttctcctcccga

SEQ ID NO: 292 - DNA, 20 bp, synthetic construct
  source 1..20: mol_type = other DNA
tcttctcctcccgatgtgcc

SEQ ID NO: 293 - DNA, 20 bp, synthetic construct
  source 1..20: mol_type = other DNA
tcctcccgatgtgccagtat

SEQ ID NO: 294 - DNA, 20 bp, synthetic construct
  source 1..20: mol_type = other DNA
ttgcaacgatagcttttgct

SEQ ID NO: 295 - DNA, 20 bp, synthetic construct
  source 1..20: mol_type = other DNA
ggttgctgtggacgtttcac

SEQ ID NO: 296 - DNA, 20 bp, synthetic construct
  source 1..20: mol_type = other DNA
tcactggccattggcttctc

SEQ ID NO: 297 - DNA, 20 bp, synthetic construct
  source 1..20: mol_type = other DNA
gtccgcctgccgagcctcaa

SEQ ID NO: 298 - DNA, 20 bp, synthetic construct
  source 1..20: mol_type = other DNA
tctcagggcttctcatctat

SEQ ID NO: 299 - DNA, 20 bp, synthetic construct
  source 1..20: mol_type = other DNA
tcatctatgatgtcttttgg

SEQ ID NO: 300 - DNA, 20 bp, synthetic construct
  source 1..20: mol_type = other DNA
aatagcaacgtcatggtgaa

SEQ ID NO: 301 - DNA, 20 bp, synthetic construct
  source 1..20: mol_type = other DNA
accatgacgttgctattgaa

SEQ ID NO: 302 - DNA, 20 bp, synthetic construct
  source 1..20: mol_type = other DNA
cgggatagaacgtcaagggg

SEQ ID NO: 303 - DNA, 20 bp, synthetic construct
  source 1..20: mol_type = other DNA
tatcccggaagctccacctg

SEQ ID NO: 304 - DNA, 20 bp, synthetic construct
  source 1..20: mol_type = other DNA
ctcgcctgtctctgcctgga

SEQ ID NO: 305 - DNA, 20 bp, synthetic construct
  source 1..20: mol_type = other DNA
tccatgttgggcatcggaga

SEQ ID NO: 306 - DNA, 20 bp, synthetic construct
  source 1..20: mol_type = other DNA
gtccttcgctatgacaacta

SEQ ID NO: 307 - DNA, 20 bp, synthetic construct
  source 1..20: mol_type = other DNA
gctatgacaactacaaaaag

SEQ ID NO: 308 - DNA, 20 bp, synthetic construct
  source 1..20: mol_type = other DNA
ttgtagttgtcatagcgaag

SEQ ID NO: 309 - DNA, 20 bp, synthetic construct
  source 1..20: mol_type = other DNA
tgcatgcgcccggagatgtt

SEQ ID NO: 310 - DNA, 20 bp, synthetic construct
  source 1..20: mol_type = other DNA
cactgcaccctcatcggata

SEQ ID NO: 311 - DNA, 20 bp, synthetic construct
  source 1..20: mol_type = other DNA
tcttacctacaaagtatccg

SEQ ID NO: 312 - DNA, 20 bp, synthetic construct
  source 1..20: mol_type = other DNA
tctatttggtgccatttact

SEQ ID NO: 313 - DNA, 20 bp, synthetic construct
  source 1..20: mol_type = other DNA
attgccactcctcacgatgg

SEQ ID NO: 314 - DNA, 20 bp, synthetic construct
  source 1..20: mol_type = other DNA
aaataggccatcgtgaggag

SEQ ID NO: 315 - DNA, 20 bp, synthetic construct
  source 1..20: mol_type = other DNA
ccactccaagtccagcagct

SEQ ID NO: 316 - DNA, 20 bp, synthetic construct
  source 1..20: mol_type = other DNA
caggaatcgggagctgctgg